European Patent Specification EP 3 967 327 B1, published January 7, 2026. Title: Trolox Peptide Conjugate and Use Thereof. Applicant: CAREGEN CO., LTD. The sequence listing filed with the application follows.

SEQUENCE LISTING (7 sequences)

SEQ ID NO: 1 - protein, 12 aa, Artificial Sequence
  SEQ. ID. NO: 1 Peptide
ELIEHGGGRPAD

SEQ ID NO: 2 - protein, 10 aa, Artificial Sequence
  SEQ. ID. NO: 2 Peptide
RQTRVQRCHC

SEQ ID NO: 3 - protein, 10 aa, Artificial Sequence
  SEQ. ID. NO: 3 Peptide
  SITE (1): N-terminal amino acid is acetylated
YKSKKGGWTH

SEQ ID NO: 4 - DNA, 20 bp, Artificial Sequence
  MSX2 forward primer
aacacaagaccaaccggaag

SEQ ID NO: 5 - DNA, 20 bp, Artificial Sequence
  MSX2 reverse primer
gcagccattttcagcttttc

SEQ ID NO: 6 - DNA, 24 bp, Artificial Sequence
  Keratin-14 forward primer
ccacctttcatcttcccaattctc

SEQ ID NO: 7 - DNA, 18 bp, Artificial Sequence
  Keratin-14 reverse primer
gtgcggatctggcggttg